European Patent Application EP 4 202 056 A1, published June 28, 2023. Title: RNA probe for mutational profiling and use thereof. Applicant: xFOREST Therapeutics Co., Ltd. The sequence listing filed with the application follows.

SEQUENCE LISTING (10 sequences)

SEQ ID NO: 1 - RNA, 36 nt, Artificial Sequence
  sequence of interest
guguaugaugaaacuacauuaaguuaacucgugcac

SEQ ID NO: 2 - DNA, 58 bp, Artificial Sequence
  reverse primer for library design 2
gaaccggaccgaagcccgatttggagcggaagccgctcaccgttgaccagttgtgcac

SEQ ID NO: 3 - DNA, 58 bp, Artificial Sequence
  reverse primer for library design 2
gaaccggaccgaagcccgatttgggccacaaggtggccaccgttgaccagttgtgcac

SEQ ID NO: 4 - DNA, 60 bp, Artificial Sequence
  reverse primer for library design 2
gaaccggaccgaagcccgatttgacctctgttacagaggtaccgttgaccagttgtgcac

SEQ ID NO: 5 - DNA, 60 bp, Artificial Sequence
  reverse primer for library design 2
gaaccggaccgaagcccgatttgacacaccttaggtgtgtaccgttgaccagttgtgcac

SEQ ID NO: 6 - DNA, 18 bp, Artificial Sequence
  T7 RNA Polymerase promoter sequence
taatacgactcactatag

SEQ ID NO: 7 - RNA, 58 nt, Artificial Sequence
  RNA probe ID 1 with a structured barcode sequence
  misc_feature (1)..(18): structured barcode sequence
  misc_feature (21)..(56): analyte RNA sequence
guacucugagaagagugcaaguguaugaugaaacuacauuaaguuaacucgugcacaa

SEQ ID NO: 8 - RNA, 55 nt, Artificial Sequence
  RNA probe ID32  with an unstructured barcode sequence
  misc_feature (1)..(15): unstructured barcode sequence
  misc_feature (18)..(53): analyte RNA sequence
gaugucgggaugaaaaaguguaugaugaaacuacauuaaguuagcucgugcacaa

SEQ ID NO: 9 - RNA, 22 nt, Artificial Sequence
  Structured RNA barcode ID12
gcuagaagauuugucuucuggu

SEQ ID NO: 10 - RNA, 19 nt, Artificial Sequence
  Structured RNA barcode ID28
uugcgagauauucucgcga